European Patent Specification EP 3 737 773 B1, published April 12, 2023. Title: NOVEL PRIMERS AND USES THEREOF. Applicant: NATERA, INC. The sequence listing filed with the application follows.

SEQUENCE LISTING (9 sequences)

SEQ ID NO: 1 - DNA, 24 bp, Artificial Sequence
  source: /note="Description of Artificial Sequence: Synthetic primer"
  modified_base (21)..(24): a, c, t, g, unknown or other
acacgacgctcttccgatctnnnn

SEQ ID NO: 2 - DNA, 25 bp, Artificial Sequence
  source: /note="Description of Artificial Sequence: Synthetic primer"
  modified_base (22)..(25): a, c, t, g, unknown or other
agacgtgtgctcttccgatctnnnn

SEQ ID NO: 3 - DNA, 29 bp, Artificial Sequence
  source: /note="Description of Artificial Sequence: Synthetic oligonucleotide"
  modified_base (1)..(2): a, c, t, g, unknown or other
  modified_base (23)..(29): a, c, t, g, unknown or other
nnacacgacgctcttccgatctnnnnnnn

SEQ ID NO: 4 - DNA, 30 bp, Artificial Sequence
  source: /note="Description of Artificial Sequence: Synthetic oligonucleotide"
  modified_base (1)..(7): a, c, t, g, unknown or other
  modified_base (29)..(30): a, c, t, g, unknown or other
nnnnnnnagatcggaagagcacacgtctnn

SEQ ID NO: 5 - DNA, 28 bp, Artificial Sequence
  source: /note="Description of Artificial Sequence: Synthetic primer"
  modified_base (23)..(26): a, c, t, g, unknown or other
ggacacgacgctcttccgatctnnnncc

SEQ ID NO: 6 - DNA, 29 bp, Artificial Sequence
  source: /note="Description of Artificial Sequence: Synthetic primer"
  modified_base (24)..(27): a, c, t, g, unknown or other
ggagacgtgtgctcttccgatctnnnncc

SEQ ID NO: 7 - DNA, 33 bp, Artificial Sequence
  source: /note="Description of Artificial Sequence: Synthetic oligonucleotide"
  modified_base (1)..(2): a, c, t, g, unknown or other
  modified_base (25)..(28): a, c, t, g, unknown or other
  modified_base (31)..(33): a, c, t, g, unknown or other
nnggacacgacgctcttccgatctnnnnccnnn

SEQ ID NO: 8 - DNA, 34 bp, Artificial Sequence
  source: /note="Description of Artificial Sequence: Synthetic oligonucleotide"
  modified_base (1)..(3): a, c, t, g, unknown or other
  modified_base (6)..(9): a, c, t, g, unknown or other
  modified_base (33)..(34): a, c, t, g, unknown or other
nnnggnnnnagatcggaagagcacacgtctccnn

SEQ ID NO: 9 - DNA, 28 bp, Artificial Sequence
  source: /note="Description of Artificial Sequence: Synthetic oligonucleotide"
  modified_base (1)..(2): a, c, t, g, unknown or other
  modified_base (23)..(28): a, c, t, g, unknown or other
nnacacgacgctcttccgatctnnnnnn